European Patent Application EP 4 814 021 A1, published September 30, 2026. Title: 抗体の分析方法. Applicant: CHUGAI SEIYAKU KABUSHIKI KAISHA. The sequence listing filed with the application follows.

SEQUENCE LISTING (86 sequences)

SEQ ID NO: 1 - protein, 330 aa, synthetic construct [sequence omitted]

SEQ ID NO: 2 - protein, 326 aa, synthetic construct
  source 1..326: note = an artificially synthesized sequence
ASTKGPSVFPLAPCSRSTSESTAALGCLVKDYFPEPVTVSWNSGALTSGVHTFPAVLQSSGLYSLSSVVTVPSSNFGTQTYTCNVDHKPSNTKVDKTVERKCCVECPPCPAPPVAGPSVFLFPPKPKDTLMISRTPEVTCVVVDVSHEDPEVQFNWYVDGVEVHNAKTKPREEQFNSTFRVVSVLTVVHQDWLNGKEYKCKVSNKGLPAPIEKTISKTKGQPREPQVYTLPPSREEMTKNQVSLTCLVKGFYPSDIAVEWESNGQPENNYKTTPPMLDSDGSFFLYSKLTVDKSRWQQGNVFSCSVMHEALHNHYTQKSLSLSPGK

SEQ ID NO: 3 - protein, 377 aa, synthetic construct
  source 1..377: note = an artificially synthesized sequence
ASTKGPSVFPLAPCSRSTSGGTAALGCLVKDYFPEPVTVSWNSGALTSGVHTFPAVLQSSGLYSLSSVVTVPSSSLGTQTYTCNVNHKPSNTKVDKRVELKTPLGDTTHTCPRCPEPKSCDTPPPCPRCPEPKSCDTPPPCPRCPEPKSCDTPPPCPRCPAPELLGGPSVFLFPPKPKDTLMISRTPEVTCVVVDVSHEDPEVQFKWYVDGVEVHNAKTKPREEQYNSTFRVVSVLTVLHQDWLNGKEYKCKVSNKALPAPIEKTISKTKGQPREPQVYTLPPSREEMTKNQVSLTCLVKGFYPSDIAVEWESSGQPENNYNTTPPMLDSDGSFFLYSKLTVDKSRWQQGNIFSCSVMHEALHNRFTQKSLSLSPGK

SEQ ID NO: 4 - protein, 327 aa, synthetic construct
  source 1..327: note = an artificially synthesized sequence
ASTKGPSVFPLAPCSRSTSESTAALGCLVKDYFPEPVTVSWNSGALTSGVHTFPAVLQSSGLYSLSSVVTVPSSSLGTKTYTCNVDHKPSNTKVDKRVESKYGPPCPSCPAPEFLGGPSVFLFPPKPKDTLMISRTPEVTCVVVDVSQEDPEVQFNWYVDGVEVHNAKTKPREEQFNSTYRVVSVLTVLHQDWLNGKEYKCKVSNKGLPSSIEKTISKAKGQPREPQVYTLPPSQEEMTKNQVSLTCLVKGFYPSDIAVEWESNGQPENNYKTTPPVLDSDGSFFLYSRLTVDKSRWQEGNVFSCSVMHEALHNHYTQKSLSLSLGK

SEQ ID NO: 5 - protein, 4 aa, synthetic construct
  source 1..4: note = an artificially synthesized sequence
GGGS

SEQ ID NO: 6 - protein, 4 aa, synthetic construct
  source 1..4: note = an artificially synthesized sequence
SGGG

SEQ ID NO: 7 - protein, 5 aa, synthetic construct
  source 1..5: note = an artificially synthesized sequence
GGGGS

SEQ ID NO: 8 - protein, 5 aa, synthetic construct
  source 1..5: note = an artificially synthesized sequence
SGGGG

SEQ ID NO: 9 - protein, 6 aa, synthetic construct
  source 1..6: note = an artificially synthesized sequence
GGGGGS

SEQ ID NO: 10 - protein, 6 aa, synthetic construct
  source 1..6: note = an artificially synthesized sequence
SGGGGG

SEQ ID NO: 11 - protein, 7 aa, synthetic construct
  source 1..7: note = an artificially synthesized sequence
GGGGGGS

SEQ ID NO: 12 - protein, 7 aa, synthetic construct
  source 1..7: note = an artificially synthesized sequence
SGGGGGG

SEQ ID NO: 13 - protein, 207 aa, synthetic construct
  source 1..207: note = an artificially synthesized sequence
MQSGTHWRVLGLCLLSVGVWGQDGNEEMGGITQTPYKVSISGTTVILTCPQYPGSEILWQHNDKNIGGDEDDKNIGSDEDHLSLKEFSELEQSGYYVCYPRGSKPEDANFYLYLRARVCENCMEMDVMSVATIVIVDICITGGLLLLVYYWSKNRKAKAKPVTRGAGAGGRQRGQNKERPPPVPNPDYEPIRKGQRDLYSGLNQRRI

SEQ ID NO: 14 - protein, 72 aa, synthetic construct
  source 1..72: note = an artificially synthesized sequence
SPCPPNSFSSAGGQRTCDICRQCKGVFRTRKECSSTSNAECDCTPGFHCLGAGCSMCEQDCKQGQELTKKGC

SEQ ID NO: 15 - protein, 31 aa, synthetic construct
  source 1..31: note = an artificially synthesized sequence
DCTPGFHCLGAGCSMCEQDCKQGQELTKKGC

SEQ ID NO: 16 - protein, 63 aa, synthetic construct
  source 1..63: note = an artificially synthesized sequence
LQDPCSNCPAGTFCDNNRNQICSPCPPNSFSSAGGQRTCDICRQCKGVFRTRKECSSTSNAEC

SEQ ID NO: 17 - protein, 22 aa, synthetic construct
  source 1..22: note = an artificially synthesized sequence
LQDPCSNCPAGTFCDNNRNQIC

SEQ ID NO: 18 - protein, 11 aa, synthetic construct
  source 1..11: note = an artificially synthesized sequence
VEPKSCGGGGS

SEQ ID NO: 19 - protein, 16 aa, synthetic construct
  source 1..16: note = an artificially synthesized sequence
VEPKSCGGGGSGGGGS

SEQ ID NO: 20 - protein, 6 aa, synthetic construct
  source 1..6: note = an artificially synthesized sequence
VEPKSC

SEQ ID NO: 21 - protein, 88 aa, synthetic construct
  source 1..88: note = an artificially synthesized sequence
MVLASSTTSIHTMLLLLLMLAQPAMARADPCAARPCAHGGRCYAHFSGLVCACAPGYMGARCEFPVHPDGASALPAAPPGLRPGDPQR

SEQ ID NO: 22 - protein, 618 aa, synthetic construct
  source 1..618: note = an artificially synthesized sequence
MVSPRMSGLLSQTVILALIFLPQTRPAGVFELQIHSFGPGPGPGAPRSPCSARLPCRLFFRVCLKPGLSEEAAESPCALGAALSARGPVYTEQPGAPAPDLPLPDGLLQVPFRDAWPGTFSFIIETWREELGDQIGGPAWSLLARVAGRRRLAAGGPWARDIQRAGAWELRFSYRARCEPPAVGTACTRLCRPRSAPSRCGPGLRPCAPLEDECEAPLVCRAGCSPEHGFCEQPGECRCLEGWTGPLCTVPVSTSSCLSPRGPSSATTGCLVPGPGPCDGNPCANGGSCSETPRSFECTCPRGFYGLRCEVSGVTCADGPCFNGGLCVGGADPDSAYICHCPPGFQGSNCEKRVDRCSLQPCRNGGLCLDLGHALRCRCRAGFAGPRCEHDLDDCAGRACANGGTCVEGGGAHRCSCALGFGGRDCRERADPCAARPCAHGGRCYAHFSGLVCACAPGYMGARCEFPVHPDGASALPAAPPGLRPGDPQRYLLPPALGLLVAAGVAGAALLLVHVRRRGHSQDAGSRLLAGTPEPSVHALPDALNNLRTQEGSGDGPSSSVDWNRPEDVDPQGIYVISAPSIYAREVATPLFPPLHTGRAGQRQHLLFPYPSSILSVK

SEQ ID NO: 23 - protein, 220 aa, synthetic construct
  source 1..220: note = an artificially synthesized sequence
CPPCPAPEAAGGPSVFLFPPKPKDTLMISRTPEVTCVVVDVSHEDPEVKFNWYVDGVEVHNAKTKPREEQYASTYRVVSVLTVLHQDWLNGKEYKCKVSNKALPAPIEKTISKAKGQPREPQVYTLPPCRDELTKNQVSLWCLVKGFYPSDIAVEWESNGQPENNYKTTPPVLDSDGSFFLYSKLTVDKSRWQQGNVFSCSVLHEALHAHYTRKELSLSP

SEQ ID NO: 24 - protein, 220 aa, synthetic construct
  source 1..220: note = an artificially synthesized sequence
CPPCPAPEAAGGPSVFLFPPKPKDTLMISRTPEVTCVVVDVSHEDPEVKFNWYVDGVEVHNAKTKPREEQYASTYRVVSVLTVLHQDWLNGKEYKCKVSNKALPAPIEKTISKAKGQPREPQVCTLPPSRDELTKNQVSLSCAVKGFYPSDIAVEWESNGQPENNYKTTPPVLDSDGSFFLVSKLTVDKSRWQQGNVFSCSVLHEALHAHYTRKELSLSP

SEQ ID NO: 25 - protein, 220 aa, synthetic construct
  source 1..220: note = an artificially synthesized sequence
CPPCPAPEAAGGPSVFLFPPKPKDTLMISRTPEVTCVVVDVSHEDPEVKFNWYVDGVEVHNAKTKPREEQYASTYRVVSVLTVLHQDWLNGKEYKCKVSNKALPAPIEKTISKAKGQPREPQVYTLPPCRDELTKNQVSLWCLVKGFYPSDIAVEWESNGQPENNYKTTPPVLDSDGSFFLYSKLTVDKSRWQEGNVFSCSVLHEALHAHYTRKELSLSP

SEQ ID NO: 26 - protein, 220 aa, synthetic construct
  source 1..220: note = an artificially synthesized sequence
CPPCPAPEAAGGPSVFLFPPKPKDTLMISRTPEVTCVVVDVSHEDPEVKFNWYVDGVEVHNAKTKPREEQYASTYRVVSVLTVLHQDWLNGKEYKCKVSNKALPAPIEKTISKAKGQPREPQVCTLPPSRDELTKNQVSLSCAVKGFYPSDIAVEWESNGQPENNYKTTPPVLDSDGSFFLVSKLTVDKSRWQEGNVFSCSVLHEALHAHYTRKELSLSP

SEQ ID NO: 27 - protein, 5 aa, synthetic construct
  source 1..5: note = an artificially synthesized sequence
NVWFH

SEQ ID NO: 28 - protein, 19 aa, synthetic construct
  source 1..19: note = an artificially synthesized sequence
QIKDYYNAYAAYYAPSVKG

SEQ ID NO: 29 - protein, 17 aa, synthetic construct
  source 1..17: note = an artificially synthesized sequence
VHYASASTLLPAEGVDA

SEQ ID NO: 30 - protein, 16 aa, synthetic construct
  source 1..16: note = an artificially synthesized sequence
QPSQEVVHMNRNTYLH

SEQ ID NO: 31 - protein, 7 aa, synthetic construct
  source 1..7: note = an artificially synthesized sequence
KVSNRFP

SEQ ID NO: 32 - protein, 9 aa, synthetic construct
  source 1..9: note = an artificially synthesized sequence
AQGTSHPFT

SEQ ID NO: 33 - protein, 5 aa, synthetic construct
  source 1..5: note = an artificially synthesized sequence
NVWFH

SEQ ID NO: 34 - protein, 19 aa, synthetic construct
  source 1..19: note = an artificially synthesized sequence
QIKDYYNAYAGYYHPSVKG

SEQ ID NO: 35 - protein, 17 aa, synthetic construct
  source 1..17: note = an artificially synthesized sequence
VHYAAASQLLPAEGVDA

SEQ ID NO: 36 - protein, 128 aa, synthetic construct
  source 1..128: note = an artificially synthesized sequence
QVQLVESGGGLVQPGRSLRLSCAASGFKFSNVWFHWVRQAPGKGLEWVAQIKDYYNAYAAYYAPSVKGRFTISRDDSKNSIYLQMNSLKTEDTAVYYCHYVHYASASTLLPAEGVDAWGQGTTVTVSS

SEQ ID NO: 37 - protein, 112 aa, synthetic construct
  source 1..112: note = an artificially synthesized sequence
DIVMTQSPLSLPVTPGEPASISCQPSQEVVHMNRNTYLHWYQQKPGQAPRLLIYKVSNRFPGVPDRFSGSGSGTDFTLKISRVEAEDVGVYYCAQGTSHPFTFGQGTKLEIK

SEQ ID NO: 38 - protein, 128 aa, synthetic construct
  source 1..128: note = an artificially synthesized sequence
QVQLVESGGGLVQPGRSLRLSCAASGFKFSNVWFHWVRQAPGKGLEWVAQIKDYYNAYAGYYHPSVKGRFTISRDDSKNSIYLQMNSLKTEDTAVYYCHYVHYAAASQLLPAEGVDAWGQGTTVTVSS

SEQ ID NO: 39 - protein, 681 aa, synthetic construct
  source 1..681: note = an artificially synthesized sequence
DIQLTQSPSFLSASVGDRVTITCQSTESVYGSDWLSWYQQKPGQPPKLLIYQASNLEIGVPSRFSGSGSGTDFTLTINSLEAEDAATYYCQGYYSGYIYAFGGGTKVEIKSSASTKGPSVFPLAPSSRSTSESTAALGCLVKDYFPEPVTVSWNSGALTSGVHTFPAVLQSSGLYSLSSVVTVPSSSLGTKTYTCNVDHKPSNTKVDKRVEPKSCGGGGSGGGGSQVQLVESGGGLVQPGRSLRLSCAASGFKFSNVWFHWVRQAPGKGLEWVAQIKDYYNAYAAYYAPSVKGRFTISRDDSKNSIYLQMNSLKTEDTAVYYCHYVHYASASTLLPAEGVDAWGQGTTVTVSSASTKGPSVFPLAPSSKSTSGGTAALGCLVEDYFPEPVTVSWNSGALTSGVHTFPAVLQSSGLYSLSSVVTVPSCSLGTQTYICNVNHKPSNTKVDEKVEPKSCDKTHTCPPCPAPEAAGGPSVFLFPPKPKDTLMISRTPEVTCVVVDVSHEDPEVKFNWYVDGVEVHNAKTKPREEQYASTYRVVSVLTVLHQDWLNGKEYKCKVSNKALPAPIEKTISKAKGQPREPQVYTLPPCRDELTKNQVSLWCLVKGFYPSDIAVEWESNGQPENNYKTTPPVLDSDGSFFLYSKLTVDKSRWQEGNVFSCSVLHEALHAHYTRKELSLSP

SEQ ID NO: 40 - protein, 226 aa, synthetic construct
  source 1..226: note = an artificially synthesized sequence
QVTLRESGPALVKPTQTLTLTCTFSGFSLSSSYDMGWVRQAPGQGLEWMGTIYTGDYSTDYASWAKGRVTISVDRSKNQFSLKLSSVTAADTAVYYCARHTGYGYFGLWGQGTLVTVSSASVAAPSVFIFPPSDEQLKSGTASVVCLLNNFYPREAKVQWKVDNALQSGNSQESVTEQDSKDSTYSLSSTLTLSKADYEKHKVYACEVTHQGLSSPVTKSFNRGEC

SEQ ID NO: 41 - protein, 456 aa, synthetic construct
  source 1..456: note = an artificially synthesized sequence
QVQLVESGGGLVQPGRSLRLSCAASGFKFSNVWFHWVRQAPGKGLEWVAQIKDYYNAYAAYYAPSVKGRFTISRDDSKNSIYLQMNSLKTEDTAVYYCHYVHYASASTLLPAEGVDAWGQGTTVTVSSASTKGPSVFPLAPSSKSTSGGTAALGCLVEDYFPEPVTVSWNSGALTSGVHTFPAVLQSSGLYSLSSVVTVPSCSLGTQTYICNVNHKPSNTKVDEKVEPKSCDKTHTCPPCPAPEAAGGPSVFLFPPKPKDTLMISRTPEVTCVVVDVSHEDPEVKFNWYVDGVEVHNAKTKPREEQYASTYRVVSVLTVLHQDWLNGKEYKCKVSNKALPAPIEKTISKAKGQPREPQVCTLPPSRDELTKNQVSLSCAVKGFYPSDIAVEWESNGQPENNYKTTPPVLDSDGSFFLVSKLTVDKSRWQEGNVFSCSVLHEALHAHYTRKELSLSP

SEQ ID NO: 42 - protein, 219 aa, synthetic construct
  source 1..219: note = an artificially synthesized sequence
DIVMTQSPLSLPVTPGEPASISCQPSQEVVHMNRNTYLHWYQQKPGQAPRLLIYKVSNRFPGVPDRFSGSGSGTDFTLKISRVEAEDVGVYYCAQGTSHPFTFGQGTKLEIKRTVAAPSVFIFPPSDRKLKSGTASVVCLLNNFYPREAKVQWKVDNALQSGNSQESVTEQDSKDSTYSLSSTLTLSKADYEKHKVYACEVTHQGLSSPVTKSFNRGEC

SEQ ID NO: 43 - protein, 681 aa, synthetic construct
  source 1..681: note = an artificially synthesized sequence
DIQLTQSPSFLSASVGDRVTITCQSTESVYGSDWLSWYQQKPGQPPKLLIYQASNLEIGVPSRFSGSGSGTDFTLTINSLEAEDAATYYCQGYYSGYIYAFGGGTKVEIKSSASTKGPSVFPLAPSSRSTSESTAALGCLVKDYFPEPVTVSWNSGALTSGVHTFPAVLQSSGLYSLSSVVTVPSSSLGTKTYTCNVDHKPSNTKVDKRVEPKSCGGGGSGGGGSQVQLVESGGGLVQPGRSLRLSCAASGFKFSNVWFHWVRQAPGKGLEWVAQIKDYYNAYAAYYAPSVKGRFTISRDDSKNSIYLQMNSLKTEDTAVYYCHYVHYASASTLLPAEGVDAWGQGTTVTVSSASTKGPSVFPLAPSSKSTSGGTAALGCLVEDYFPEPVTVSWNSGALTSGVHTFPAVLQSSGLYSLSSVVTVPSCSLGTQTYICNVNHKPSNTKVDEKVEPKSCDKTHTCPPCPAPEAAGGPSVFLFPPKPKDTLMISRTPEVTCVVVDVSHEDPEVKFNWYVDGVEVHNAKTKPREEQYASTYRVVSVLTVLHQDWLNGKEYKCKVSNKALPAPIEKTISKAKGQPREPQVYTLPPCRDELTKNQVSLWCLVKGFYPSDIAVEWESNGQPENNYKTTPPVLDSDGSFFLYSKLTVDKSRWQQGNVFSCSVLHEALHAHYTRKELSLSP

SEQ ID NO: 44 - protein, 456 aa, synthetic construct
  source 1..456: note = an artificially synthesized sequence
QVQLVESGGGLVQPGRSLRLSCAASGFKFSNVWFHWVRQAPGKGLEWVAQIKDYYNAYAAYYAPSVKGRFTISRDDSKNSIYLQMNSLKTEDTAVYYCHYVHYASASTLLPAEGVDAWGQGTTVTVSSASTKGPSVFPLAPSSKSTSGGTAALGCLVEDYFPEPVTVSWNSGALTSGVHTFPAVLQSSGLYSLSSVVTVPSCSLGTQTYICNVNHKPSNTKVDEKVEPKSCDKTHTCPPCPAPEAAGGPSVFLFPPKPKDTLMISRTPEVTCVVVDVSHEDPEVKFNWYVDGVEVHNAKTKPREEQYASTYRVVSVLTVLHQDWLNGKEYKCKVSNKALPAPIEKTISKAKGQPREPQVCTLPPSRDELTKNQVSLSCAVKGFYPSDIAVEWESNGQPENNYKTTPPVLDSDGSFFLVSKLTVDKSRWQQGNVFSCSVLHEALHAHYTRKELSLSP

SEQ ID NO: 45 - protein, 676 aa, synthetic construct
  source 1..676: note = an artificially synthesized sequence
DIQLTQSPSFLSASVGDRVTITCQSTESVYGSDWLSWYQQKPGQPPKLLIYQASNLEIGVPSRFSGSGSGTDFTLTINSLEAEDAATYYCQGYYSGYIYAFGGGTKVEIKSSASTKGPSVFPLAPSSRSTSESTAALGCLVKDYFPEPVTVSWNSGALTSGVHTFPAVLQSSGLYSLSSVVTVPSSSLGTKTYTCNVDHKPSNTKVDKRVEPKSCGGGGSQVQLVESGGGLVQPGRSLRLSCAASGFKFSNVWFHWVRQAPGKGLEWVAQIKDYYNAYAAYYAPSVKGRFTISRDDSKNSIYLQMNSLKTEDTAVYYCHYVHYASASTLLPAEGVDAWGQGTTVTVSSASTKGPSVFPLAPSSKSTSGGTAALGCLVEDYFPEPVTVSWNSGALTSGVHTFPAVLQSSGLYSLSSVVTVPSCSLGTQTYICNVNHKPSNTKVDEKVEPKSCDKTHTCPPCPAPEAAGGPSVFLFPPKPKDTLMISRTPEVTCVVVDVSHEDPEVKFNWYVDGVEVHNAKTKPREEQYASTYRVVSVLTVLHQDWLNGKEYKCKVSNKALPAPIEKTISKAKGQPREPQVYTLPPCRDELTKNQVSLWCLVKGFYPSDIAVEWESNGQPENNYKTTPPVLDSDGSFFLYSKLTVDKSRWQQGNVFSCSVLHEALHAHYTRKELSLSP

SEQ ID NO: 46 - protein, 6 aa, synthetic construct
  source 1..6: note = an artificially synthesized sequence
SSYDMG

SEQ ID NO: 47 - protein, 17 aa, synthetic construct
  source 1..17: note = an artificially synthesized sequence
TIYTGDYSTDYASWAKG

SEQ ID NO: 48 - protein, 9 aa, synthetic construct
  source 1..9: note = an artificially synthesized sequence
HTGYGYFGL

SEQ ID NO: 49 - protein, 13 aa, synthetic construct
  source 1..13: note = an artificially synthesized sequence
QSTESVYGSDWLS

SEQ ID NO: 50 - protein, 7 aa, synthetic construct
  source 1..7: note = an artificially synthesized sequence
QASNLEI

SEQ ID NO: 51 - protein, 10 aa, synthetic construct
  source 1..10: note = an artificially synthesized sequence
QGYYSGYIYA

SEQ ID NO: 52 - protein, 119 aa, synthetic construct
  source 1..119: note = an artificially synthesized sequence
QVTLRESGPALVKPTQTLTLTCTFSGFSLSSSYDMGWVRQAPGQGLEWMGTIYTGDYSTDYASWAKGRVTISVDRSKNQFSLKLSSVTAADTAVYYCARHTGYGYFGLWGQGTLVTVSS

SEQ ID NO: 53 - protein, 110 aa, synthetic construct
  source 1..110: note = an artificially synthesized sequence
DIQLTQSPSFLSASVGDRVTITCQSTESVYGSDWLSWYQQKPGQPPKLLIYQASNLEIGVPSRFSGSGSGTDFTLTINSLEAEDAATYYCQGYYSGYIYAFGGGTKVEIK

SEQ ID NO: 54 - protein, 698 aa, synthetic construct
  source 1..698: note = Ab2-chain1_split
MDMRVPAQLLGLLLLWLPGARCDIQLTQSPSFLSASVGDRVTITCQSTESVYGSDWLSWYQQKPGQPPKLLIYQASNLEIGVPSRFSGSGSGTDFTLTINSLEAEDAATYYCQGYYSGYIYAFGGGTKVEIKSSASTKGPSVFPLAPSSRSTSESTAALGCLVKDYFPEPVTVSWNSGALTSGVHTFPAVLQSSGLYSLSSVVTVPSSSLGTKTYTCNVDHKPSNTKVDKRVEPKSCGGGGSQVQLVESGGGLVQPGRSLRLSCAASGFKFSNVWFHWVRQAPGKGLEWVAQIKDYYNAYAAYYAPSVKGRFTISRDDSKNSIYLQMNSLKTEDTAVYYCHYVHYASASTLLPAEGVDAWGQGTTVTVSSASTKGPSVFPLAPSSKSTSGGTAALGCLVEDYFPEPVTVSWNSGALTSGVHTFPAVLQSSGLYSLSSVVTVPSCSLGTQTYICNVNHKPSNTKVDEKVEPKSCDKTHTCPPCPAPEAAGGPSVFLFPPKPKDTLMISRTPEVTCVVVDVSHEDPEVKFNWYVDGVEVHNAKTKPREEQYASTYRVVSVLTVLHQDWLNGKEYKCKVSNKALPAPIEKTISKAKGQPREPQVYTLPPCRDELTKNQVSLWCLVKGFYPSDIAVEWESNGQPENNYKTTPPVLDSDGSFFLYSKLTVDKSRWQQGNVFSCSVLHEALHAHYTRKELSLSP

SEQ ID NO: 55 - protein, 245 aa, synthetic construct
  source 1..245: note = chain2
MGWSCIILFLVATATGVHSQVTLRESGPALVKPTQTLTLTCTFSGFSLSSSYDMGWVRQAPGQGLEWMGTIYTGDYSTDYASWAKGRVTISVDRSKNQFSLKLSSVTAADTAVYYCARHTGYGYFGLWGQGTLVTVSSASVAAPSVFIFPPSDEQLKSGTASVVCLLNNFYPREAKVQWKVDNALQSGNSQESVTEQDSKDSTYSLSSTLTLSKADYEKHKVYACEVTHQGLSSPVTKSFNRGEC

SEQ ID NO: 56 - protein, 475 aa, synthetic construct
  source 1..475: note = chain3
MGWSCIILFLVATATGVHSQVQLVESGGGLVQPGRSLRLSCAASGFKFSNVWFHWVRQAPGKGLEWVAQIKDYYNAYAAYYAPSVKGRFTISRDDSKNSIYLQMNSLKTEDTAVYYCHYVHYASASTLLPAEGVDAWGQGTTVTVSSASTKGPSVFPLAPSSKSTSGGTAALGCLVEDYFPEPVTVSWNSGALTSGVHTFPAVLQSSGLYSLSSVVTVPSCSLGTQTYICNVNHKPSNTKVDEKVEPKSCDKTHTCPPCPAPEAAGGPSVFLFPPKPKDTLMISRTPEVTCVVVDVSHEDPEVKFNWYVDGVEVHNAKTKPREEQYASTYRVVSVLTVLHQDWLNGKEYKCKVSNKALPAPIEKTISKAKGQPREPQVCTLPPSRDELTKNQVSLSCAVKGFYPSDIAVEWESNGQPENNYKTTPPVLDSDGSFFLVSKLTVDKSRWQQGNVFSCSVMHEALHNHYTQKSLSLSP

SEQ ID NO: 57 - protein, 238 aa, synthetic construct
  source 1..238: note = chain4
MGWSCIILFLVATATGVHSDIVMTQSPLSLPVTPGEPASISCQPSQEVVHMNRNTYLHWYQQKPGQAPRLLIYKVSNRFPGVPDRFSGSGSGTDFTLKISRVEAEDVGVYYCAQGTSHPFTFGQGTKLEIKRTVAAPSVFIFPPSDRKLKSGTASVVCLLNNFYPREAKVQWKVDNALQSGNSQESVTEQDSKDSTYSLSSTLTLSKADYEKHKVYACEVTHQGLSSPVTKSFNRGEC

SEQ ID NO: 58 - protein, 216 aa, synthetic construct
  source 1..216: note = Ab2-chain1_split_Fc
PAPEAAGGPSVFLFPPKPKDTLMISRTPEVTCVVVDVSHEDPEVKFNWYVDGVEVHNAKTKPREEQYASTYRVVSVLTVLHQDWLNGKEYKCKVSNKALPAPIEKTISKAKGQPREPQVYTLPPCRDELTKNQVSLWCLVKGFYPSDIAVEWESNGQPENNYKTTPPVLDSDGSFFLYSKLTVDKSRWQQGNVFSCSVLHEALHAHYTRKELSLSP

SEQ ID NO: 59 - protein, 216 aa, synthetic construct
  source 1..216: note = chain3_Fc
PAPEAAGGPSVFLFPPKPKDTLMISRTPEVTCVVVDVSHEDPEVKFNWYVDGVEVHNAKTKPREEQYASTYRVVSVLTVLHQDWLNGKEYKCKVSNKALPAPIEKTISKAKGQPREPQVCTLPPSRDELTKNQVSLSCAVKGFYPSDIAVEWESNGQPENNYKTTPPVLDSDGSFFLVSKLTVDKSRWQQGNVFSCSVMHEALHNHYTQKSLSLSP

SEQ ID NO: 60 - protein, 475 aa, synthetic construct
  source 1..475: note = chain3
MGWSCIILFLVATATGVHSQVQLVESGGGLVQPGRSLRLSCAASGFKFSNVWFHWVRQAPGKGLEWVAQIKDYYNAYAAYYAPSVKGRFTISRDDSKNSIYLQMNSLKTEDTAVYYCHYVHYASASTLLPAEGVDAWGQGTTVTVSSASTKGPSVFPLAPSSKSTSGGTAALGCLVEDYFPEPVTVSWNSGALTSGVHTFPAVLQSSGLYSLSSVVTVPSCSLGTQTYICNVNHKPSNTKVDEKVEPKSCDKTHTCPPCPAPEAAGGPSVFLFPPKPKDTLMISRTPEVTCVVVDVSHEDPEVKFNWYVDGVEVHNAKTKPREEQYASTYRVVSVLTVLHQDWLNGKEYKCKVSNKALPAPIEKTISKAKGQPREPQVCTLPPSRDELTKNQVSLSCAVKGFYPSDIAVEWESNGQPENNYKTTPPVLDSDGSFFLVSKLTVDKSRWQQGNVFSCSVLHEALHAHYTRKELSLSP

SEQ ID NO: 61 - protein, 586 aa, Streptococcus agalactiae
NQNNIQETNLVEKNSEDKFIQELNRYKTEIPNFKGFNVWILGDKGYYKNLINLEEIKNIQATLKKERNEEYVFVKLNGKIAHDTTVFLMNKKHKLLKNIEEFKTITQKRLTERGKFPYDTVHSTFEIKDENFIMERLKSSGLSMGKPVDYMGVNGIPIYTKTLSIDNKFAFENNSKDSSYSSNINISEDKIKENDQKILDLIVKSGANNQNLTDEEKVIAFTKYIGEITNYDNEAYRARNVDTEYYRASDLFSVTERKLAMCVGYSVTAARAFNIMGIPSYVVSGKSPQGISHAAVRAYYNRSWHIIDITASTYWKNGNYKTTYSDFIKEYCIDGYDVYDPAKTNNRFKVKYMESNEAFENWIHNNGSKSMLFINESAALKDKKPKDDFVPVTEKEKNELIDKYKKLLSQIPENTQNPGEKNIRDYLKNEYEEILKKDNLFEHEHAEFKESLNLNESFYLQLKKEEKKPSDNLKKEEKPRENSVKERETPAENNDFVSVTEKNNLIDKYKELLSKIPENTQNPGEKNIRNYLEKEYEELLQKDKLFKHEYTEFTKSLNLNETFYSQLKEGEMKLSENPEKGETNTN

SEQ ID NO: 62 - DNA, 1761 bp, Streptococcus agalactiae
  source 1..1761: mol_type = genomic DNA
aatcaaaataatattcaagaaactaatctagttgaaaaaaacagtgaagataagtttattcaagagttaaataggtataaaacagagataccaaatttcaaaggttttaatgtttggattttaggtgataaaggttattacaaaaaccttatcaatttagaagaaattaaaaatatccaagctacattaaaaaaagaaagaaatgaagaatatgtctttgtcaaattaaatgggaaaatcgcacatgatacaacagtattcttgatgaataaaaaacataaattacttaaaaatatagaggaatttaagacgataacccaaaaaaggctaactgagagaggaaagttcccatatgataccgttcattctacgtttgaaattaaggatgaaaactttatcatggaaagattgaaatcatcagggttatctatgggtaaaccagttgattatatgggcgtaaatggtatccctatttacactaaaacattatctatagataataagtttgcctttgaaaataattcaaaagattcttcatattcttcaaacattaatattagtgaagataaaataaaagaaaatgaccaaaaaattctagatttaatagttaaatctggagctaataatcaaaacttaacagatgaagaaaaagtaattgctttcactaaatatataggtgaaataactaattatgacaatgaagcttacagagctagaaatgtcgacacagaatattacagagcttcagatttattttctgtaacagaaagaaaacttgctatgtgcgttggctatagtgtaacagccgctagggcatttaatattatggggatacctagttatgtcgtttctggtaaaagtcctcaaggaatatctcatgcagctgtgagagcgtattataatagaagttggcatatcatagatatcacagccagtacatattggaaaaatggtaattacaaaacaacgtattccgattttattaaagaatactgtatagatggttatgacgtttatgatcccgcaaaaacaaataatagatttaaagttaagtatatggaatcaaatgaagcgtttgaaaattggatacataataatggaagcaaatctatgttatttattaatgaatctgcagctctaaaagataaaaaaccaaaagatgattttgtaccagtaacagaaaaagaaaaaaacgagctgatagataagtataaaaaattattgtcacagattcctgaaaacacacaaaatccaggagaaaaaaacataagagattatttgaaaaatgaatatgaagaaatattaaagaaagataatttatttgagcatgaacatgcagaatttaaagaaagtctaaatttaaatgaatcattctacctacaattaaagaaagaagaaaagaaaccgagtgataatctcaaaaaagaagaaaaaccaagagaaaattcagtaaaagagagggagactccagctgaaaacaatgattttgtttcagtaacagaaaaaaacaacttgattgataaatataaagaattattatcaaaaatcccagagaatacacaaaatcctggggaaaagaatatacgaaattatctagagaaagaatatgaagaactactacaaaaagataaattattcaagcatgagtacacagagtttacaaaaagtctaaatttgaatgaaacattctattcacaattaaaagaaggagaaatgaaactaagtgaaaatcccgaaaaaggagaaacgaacacgaattag

SEQ ID NO: 63 - protein, 681 aa, synthetic construct; identical to SEQ ID NO: 43
  source 1..681: note = chain A

SEQ ID NO: 64 - protein, 226 aa, synthetic construct; identical to SEQ ID NO: 40
  source 1..226: note = chain L

SEQ ID NO: 65 - protein, 456 aa, synthetic construct; identical to SEQ ID NO: 44
  source 1..456: note = chain P

SEQ ID NO: 66 - protein, 219 aa, synthetic construct; identical to SEQ ID NO: 42
  source 1..219: note = chain S

SEQ ID NO: 67 - protein, 681 aa, synthetic construct
  source 1..681: note = chain A
DIQLTQSPSFLSASVGDRVTITCQSTESVYGSDWLSWYQQKPGQPPKLLIYQASNLEIGVPSRFSGSGSGTDFTLTINSLEAEDAATYYCQGYYSGYIYAFGGGTKVEIKSSASTKGPSVFPLAPSSRSTSESTAALGCLVKDYFPEPVTVSWNSGALTSGVHTFPAVLQSSGLYSLSSVVTVPSSSLGTKTYTCNVDHKPSNTKVDKRVEPKSCGGGGSGGGGSQVQLVESGGGLVQPGRSLRLSCAASGFKFSNVWFHWVRQAPGKGLEWVAQIKDYYNAYAAYYAPSVKGRFTISRDDSKNSIYLQMNSLKTEDTAVYYCHYVHYASASTLLPAEGVDAWGQGTTVTVSSASTKGPSVFPLAPSSKSTSGGTAALGCLVEDYFPEPVTVSWNSGALTSGVHTFPAVLQSSGLYSLSSVVTVPSSSLGTQCYICNVNHKPSNTKVDEKVEPKSCDKTHTCPPCPAPEAAGGPSVFLFPPKPKDTLMISRTPEVTCVVVDVSHEDPEVKFNWYVDGVEVHNAKTKPREEQYASTYRVVSVLTVLHQDWLNGKEYKCKVSNKALPAPIEKTISKAKGQPREPQVYTLPPCRDELTKNQVSLWCLVKGFYPSDIAVEWESNGQPENNYKTTPPVLDSDGSFFLYSKLTVDKSRWQQGNVFSCSVLHEALHAHYTRKELSLSP

SEQ ID NO: 68 - protein, 226 aa, synthetic construct; identical to SEQ ID NO: 40
  source 1..226: note = chain L

SEQ ID NO: 69 - protein, 456 aa, synthetic construct
  source 1..456: note = chain P
QVQLVESGGGLVQPGRSLRLSCAASGFKFSNVWFHWVRQAPGKGLEWVAQIKDYYNAYAAYYAPSVKGRFTISRDDSKNSIYLQMNSLKTEDTAVYYCHYVHYASASTLLPAEGVDAWGQGTTVTVSSASTKGPSVFPLAPSSKSTSGGTAALGCLVEDYFPEPVTVSWNSGALTSGVHTFPAVLQSSGLYSLSSVVTVPSSSLGTQCYICNVNHKPSNTKVDEKVEPKSCDKTHTCPPCPAPEAAGGPSVFLFPPKPKDTLMISRTPEVTCVVVDVSHEDPEVKFNWYVDGVEVHNAKTKPREEQYASTYRVVSVLTVLHQDWLNGKEYKCKVSNKALPAPIEKTISKAKGQPREPQVCTLPPSRDELTKNQVSLSCAVKGFYPSDIAVEWESNGQPENNYKTTPPVLDSDGSFFLVSKLTVDKSRWQQGNVFSCSVLHEALHAHYTRKELSLSP

SEQ ID NO: 70 - protein, 219 aa, synthetic construct; identical to SEQ ID NO: 42
  source 1..219: note = chain S

SEQ ID NO: 71 - protein, 681 aa, synthetic construct
  source 1..681: note = chain A
DIQLTQSPSFLSASVGDRVTITCQSTESVYGSDWLSWYQQKPGQPPKLLIYQASNLEIGVPSRFSGSGSGTDFTLTINSLEAEDAATYYCQGYYSGYIYAFGGGTKVEIKSSASTKGPSVFPLAPSSRSTSESTAALGCLVKDYFPEPVTVSWNSGALTSGVHTFPAVLQSSGLYSLSSVVTVPSSSLGTKTYTCNVDHKPSNTKVDKRVEPKSCGGGGSGGGGSQVQLVESGGGLVQPGRSLRLSCAASGFKFSNVWFHWVRQAPGKGLEWVAQIKDYYNAYAAYYAPSVKGRFTISRDDSKNSIYLQMNSLKTEDTAVYYCHYVHYASASTLLPAEGVDAWGQGTTVTVSSASTKGPSVFPLAPSSKSTSGGTAALGCLVEDYFPEPVTVSWNSGALTSGVHTFPAVLQSSGLYSLSSVVTVPSSSLGCQTYICNVNHKPSNTKVDEKVEPKSCDKTHTCPPCPAPEAAGGPSVFLFPPKPKDTLMISRTPEVTCVVVDVSHEDPEVKFNWYVDGVEVHNAKTKPREEQYASTYRVVSVLTVLHQDWLNGKEYKCKVSNKALPAPIEKTISKAKGQPREPQVYTLPPCRDELTKNQVSLWCLVKGFYPSDIAVEWESNGQPENNYKTTPPVLDSDGSFFLYSKLTVDKSRWQQGNVFSCSVLHEALHAHYTRKELSLSP

SEQ ID NO: 72 - protein, 226 aa, synthetic construct; identical to SEQ ID NO: 40
  source 1..226: note = chain L

SEQ ID NO: 73 - protein, 456 aa, synthetic construct
  source 1..456: note = chain P
QVQLVESGGGLVQPGRSLRLSCAASGFKFSNVWFHWVRQAPGKGLEWVAQIKDYYNAYAAYYAPSVKGRFTISRDDSKNSIYLQMNSLKTEDTAVYYCHYVHYASASTLLPAEGVDAWGQGTTVTVSSASTKGPSVFPLAPSSKSTSGGTAALGCLVEDYFPEPVTVSWNSGALTSGVHTFPAVLQSSGLYSLSSVVTVPSSSLGCQTYICNVNHKPSNTKVDEKVEPKSCDKTHTCPPCPAPEAAGGPSVFLFPPKPKDTLMISRTPEVTCVVVDVSHEDPEVKFNWYVDGVEVHNAKTKPREEQYASTYRVVSVLTVLHQDWLNGKEYKCKVSNKALPAPIEKTISKAKGQPREPQVCTLPPSRDELTKNQVSLSCAVKGFYPSDIAVEWESNGQPENNYKTTPPVLDSDGSFFLVSKLTVDKSRWQQGNVFSCSVLHEALHAHYTRKELSLSP

SEQ ID NO: 74 - protein, 219 aa, synthetic construct; identical to SEQ ID NO: 42
  source 1..219: note = chain S

SEQ ID NO: 75 - protein, 681 aa, synthetic construct
  source 1..681: note = chain A
DIQLTQSPSFLSASVGDRVTITCQSTESVYGSDWLSWYQQKPGQPPKLLIYQASNLEIGVPSRFSGSGSGTDFTLTINSLEAEDAATYYCQGYYSGYIYAFGGGTKVEIKSSASTKGPSVFPLAPSSRSTSESTAALGCLVKDYFPEPVTVSWNSGALTSGVHTFPAVLQSSGLYSLSSVVTVPSSSLGTKTYTCNVDHKPSNTKVDKRVEPKSCGGGGSGGGGSQVQLVESGGGLVQPGRSLRLSCAASGFKFSNVWFHWVRQAPGKGLEWVAQIKDYYNAYAAYYAPSVKGRFTISRDDSKNSIYLQMNSLKTEDTAVYYCHYVHYASASTLLPAEGVDAWGQGTTVTVSSASTKGPSVFPLAPSSKSTSGGTAALGCLVEDYFPEPVTVSWNSGALTSGVHTFPAVLQSSGLYSLSSVVTVPSSSLGTQTYICNVNHKPSNTKVDEKVEPKSCDKTHTCPPCPAPEAAGGPSVFLFPPKPKDTLMISRTPEVTCVVVDVSHEDPEVKFNWYVDGVEVHNAKTKPREEQYASTYRVVSVLTVLHQDWLNGKEYKCKVSNKALPAPIEKTISKAKGQPREPQVYTLPPCRDELTKNQVSLWCLVKGFYPSDIAVEWESNGQPENNYKTTPPVLDSDGSFFLYSKLTVDKSRWQQGNVFSCSVLHEALHAHYTRKELSLSP

SEQ ID NO: 76 - protein, 226 aa, synthetic construct; identical to SEQ ID NO: 40
  source 1..226: note = chain L

SEQ ID NO: 77 - protein, 456 aa, synthetic construct
  source 1..456: note = chain P
QVQLVESGGGLVQPGRSLRLSCAASGFKFSNVWFHWVRQAPGKGLEWVAQIKDYYNAYAAYYAPSVKGRFTISRDDSKNSIYLQMNSLKTEDTAVYYCHYVHYASASTLLPAEGVDAWGQGTTVTVSSASTKGPSVFPLAPSSKSTSGGTAALGCLVEDYFPEPVTVSWNSGALTSGVHTFPAVLQSSGLYSLSSVVTVPSSSLGTQTYICNVNHKPSNTKVDEKVEPKSCDKTHTCPPCPAPEAAGGPSVFLFPPKPKDTLMISRTPEVTCVVVDVSHEDPEVKFNWYVDGVEVHNAKTKPREEQYASTYRVVSVLTVLHQDWLNGKEYKCKVSNKALPAPIEKTISKAKGQPREPQVCTLPPSRDELTKNQVSLSCAVKGFYPSDIAVEWESNGQPENNYKTTPPVLDSDGSFFLVSKLTVDKSRWQQGNVFSCSVLHEALHAHYTRKELSLSP

SEQ ID NO: 78 - protein, 219 aa, synthetic construct; identical to SEQ ID NO: 42
  source 1..219: note = chain S

SEQ ID NO: 79 - protein, 456 aa, synthetic construct
  source 1..456: note = chain H
QVQLVESGGGLVQPGRSLRLSCAASGFKFSNVWFHWVRQAPGKGLEWVAQIKDYYNAYAAYYAPSVKGRFTISRDDSKNSIYLQMNSLKTEDTAVYYCHYVHYASASTLLPAEGVDAWGQGTTVTVSSASTKGPSVFPLAPSSKSTSGGTAALGCLVKDYFPEPVTVSWNSGALTSGVHTFPAVLQSSGLYSLSSVVTVPSCSLGTQTYICNVNHKPSNTKVDKKVEPKSCDKTHTCPPCPAPELLGGPSVFLFPPKPKDTLMISRTPEVTCVVVDVSHEDPEVKFNWYVDGVEVHNAKTKPREEQYNSTYRVVSVLTVLHQDWLNGKEYKCKVSNKALPAPIEKTISKAKGQPREPQVYTLPPSREEMTKNQVSLTCLVKGFYPSDIAVEWESNGQPENNYKTTPPVLDSDGSFFLYSKLTVDKSRWQQGNVFSCSVMHEALHNHYTQKSLSLSP

SEQ ID NO: 80 - protein, 219 aa, synthetic construct
  source 1..219: note = chain L
DIVMTQSPLSLPVTPGEPASISCQPSQEVVHMNRNTYLHWYQQKPGQAPRLLIYKVSNRFPGVPDRFSGSGSGTDFTLKISRVEAEDVGVYYCAQGTSHPFTFGQGTKLEIKRTVAAPSVFIFPPSDEQLKSGTASVVCLLNNFYPREAKVQWKVDNALQSGNSQESVTEQDSKDSTYSLSSTLTLSKADYEKHKVYACEVTHQGLSSPVTKSFNRGEC

SEQ ID NO: 81 - protein, 456 aa, synthetic construct
  source 1..456: note = chain H
QVQLVESGGGLVQPGRSLRLSCAASGFKFSNVWFHWVRQAPGKGLEWVAQIKDYYNAYAAYYAPSVKGRFTISRDDSKNSIYLQMNSLKTEDTAVYYCHYVHYASASTLLPAEGVDAWGQGTTVTVSSASTKGPSVFPLAPSSKSTSGGTAALGCLVKDYFPEPVTVSWNSGALTSGVHTFPAVLQSSGLYSLSSVVTVPSSSLGTQCYICNVNHKPSNTKVDKKVEPKSCDKTHTCPPCPAPELLGGPSVFLFPPKPKDTLMISRTPEVTCVVVDVSHEDPEVKFNWYVDGVEVHNAKTKPREEQYNSTYRVVSVLTVLHQDWLNGKEYKCKVSNKALPAPIEKTISKAKGQPREPQVYTLPPSREEMTKNQVSLTCLVKGFYPSDIAVEWESNGQPENNYKTTPPVLDSDGSFFLYSKLTVDKSRWQQGNVFSCSVMHEALHNHYTQKSLSLSP

SEQ ID NO: 82 - protein, 219 aa, synthetic construct; identical to SEQ ID NO: 80
  source 1..219: note = chain L

SEQ ID NO: 83 - protein, 456 aa, synthetic construct
  source 1..456: note = chain H
QVQLVESGGGLVQPGRSLRLSCAASGFKFSNVWFHWVRQAPGKGLEWVAQIKDYYNAYAAYYAPSVKGRFTISRDDSKNSIYLQMNSLKTEDTAVYYCHYVHYASASTLLPAEGVDAWGQGTTVTVSSASTKGPSVFPLAPSSKSTSGGTAALGCLVKDYFPEPVTVSWNSGALTSGVHTFPAVLQSSGLYSLSSVVTVPSSSLGCQTYICNVNHKPSNTKVDKKVEPKSCDKTHTCPPCPAPELLGGPSVFLFPPKPKDTLMISRTPEVTCVVVDVSHEDPEVKFNWYVDGVEVHNAKTKPREEQYNSTYRVVSVLTVLHQDWLNGKEYKCKVSNKALPAPIEKTISKAKGQPREPQVYTLPPSREEMTKNQVSLTCLVKGFYPSDIAVEWESNGQPENNYKTTPPVLDSDGSFFLYSKLTVDKSRWQQGNVFSCSVMHEALHNHYTQKSLSLSP

SEQ ID NO: 84 - protein, 219 aa, synthetic construct; identical to SEQ ID NO: 80
  source 1..219: note = chain L

SEQ ID NO: 85 - protein, 456 aa, synthetic construct
  source 1..456: note = chain H
QVQLVESGGGLVQPGRSLRLSCAASGFKFSNVWFHWVRQAPGKGLEWVAQIKDYYNAYAAYYAPSVKGRFTISRDDSKNSIYLQMNSLKTEDTAVYYCHYVHYASASTLLPAEGVDAWGQGTTVTVSSASTKGPSVFPLAPSSKSTSGGTAALGCLVKDYFPEPVTVSWNSGALTSGVHTFPAVLQSSGLYSLSSVVTVPSSSLGTQTYICNVNHKPSNTKVDKKVEPKSCDKTHTCPPCPAPELLGGPSVFLFPPKPKDTLMISRTPEVTCVVVDVSHEDPEVKFNWYVDGVEVHNAKTKPREEQYNSTYRVVSVLTVLHQDWLNGKEYKCKVSNKALPAPIEKTISKAKGQPREPQVYTLPPSREEMTKNQVSLTCLVKGFYPSDIAVEWESNGQPENNYKTTPPVLDSDGSFFLYSKLTVDKSRWQQGNVFSCSVMHEALHNHYTQKSLSLSP

SEQ ID NO: 86 - protein, 219 aa, synthetic construct; identical to SEQ ID NO: 80
  source 1..219: note = chain L